European Patent Application EP 4 414 378 A1, published August 14, 2024. Title: Protein for use in the treatment of complement dysregulation disorders. Applicant: Ustav organicke chemie a biochemie AV CR, v. v. i. Application EP. The sequence listing filed with the application follows.

SEQUENCE LISTING (11 sequences)

SEQ ID NO: 1 - protein, 387 aa, Trypanosoma brucei gambiense
MMKYLLVFAIIATRIPVLLVIGSEDNRVPGDKKLTKEGAAALCKMKHLADKVAKERSQELKDRTQNFAGYIEFELYRIDYWLEKLNGPKGRKDGYAKLSDSDIEKVKEIFNKAKDGITKQLPEAKKAGEEAGKLHTEVKKAAENARGQDLDDDTAKSTGLYRVLNWYCITKEERHNATPNCDGIQFRKHYLSVNRSAIDCSSTSYEENYDWSANALQVALNSWEDVKPKKLESAGSDKNCNIGQSSESHPCTMTEEWQTPYKETVEKLRELEDAYQRGKKAHDAMLGYANTAYAVNTKVEQEKPLTEVIAAAKEAGKKGAKIIIPAAAPATPTNSTKNDDSAPTEHVDRGIATNETQVEVGIDADFDSLLDATEAAEVTRRHQRTAM

SEQ ID NO: 2 - protein, 28 aa, Trypanosoma brucei gambiense
YIEFELYRIDYWLEKLNGPKGRKDGYAK

SEQ ID NO: 3 - protein, 4 aa, Trypanosoma brucei gambiense
DWSA

SEQ ID NO: 4 - protein, 13 aa, Trypanosoma brucei gambiense
NTAYAVNTKVEQE

SEQ ID NO: 5 - protein, 346 aa, synthetic construct
LLVIGSEDNRVPGDKKLTKEGAAALCKMKHLADKVAKERSQELKDRTQNFAGYIEFELYRIDYWLEKLNGPKGRKDGYAKLSDSDIKKVKEIFEKAKDGITKQLPEAKKAAEEAEKLHQEVKEAAEKARGQDLDDDTAKSTGLYRVLNWYCITKEERHNATPNCDGIQFRKHYLSVNRSAIDCSSTSYEENYDWSANALQVALNSWEDKKPKKLESAGSDKNCNIGQSSESHPCTMTEEWQTHYKETIEKLRELEEAYQRGKKAHDDMLGYANTAYAVNTKVEQEKPLSEVIAAAKEAGKKGAKIIIPAAAPATPTNSTKNDDSAPTEHVDRGIATNETQVEVGID

SEQ ID NO: 6 - protein, 237 aa, synthetic construct
YIEFELYRIDYWLEKLNGPKGRKDGYAKLSDSDIKKVKEIFEKAKDGITKQLPEAKKAAEEAEKLHQEVKEAAEKARGQDLDDDTAKSTGLYRVLNWYCITKEERHNATPNCDGIQFRKHYLSVNRSAIDCSSTSYEENYDWSANALQVALNSWEDKKPKKLESAGSDKNCNIGQSSESHPCTMTEEWQTHYKETIEKLRELEEAYQRGKKAHDDMLGYANTAYAVNTKVEQEKPLS

SEQ ID NO: 7 - protein, 365 aa, synthetic construct
MMKYLLVFAIIATRIPVLLVIGSEDNRVPGDKKLTKEGAAALCKMKHLADKVAKERSQELKDRTQNFAGYIEFELYRIDYWLEKLNGPKGRKDGYAKLSDSDIKKVKEIFEKAKDGITKQLPEAKKAAEEAEKLHQEVKEAAEKARGQDLDDDTAKSTGLYRVLNWYCITKEERHNATPNCDGIQFRKHYLSVNRSAIDCSSTSYEENYDWSANALQVALNSWEDKKPKKLESAGSDKNCNIGQSSESHPCTMTEEWQTHYKETIEKLRELEEAYQRGKKAHDDMLGYANTAYAVNTKVEQEKPLSEVIAAAKEAGKKGAKIIIPAAAPATPTNSTKNDDSAPTEHVDRGIATNETQVEVGIDAD

SEQ ID NO: 8 - protein, 286 aa, synthetic construct
SEDNRVPGDKKLTKEGAAALCKMKHLADKVAKERSQELKDRTQNFAGYIEFELYRIDYWLEKLNGPKGRKDGYAKLSDSDIKKVKEIFEKAKDGITKQLPEAKKAAEEAEKLHQEVKEAAEKARGQDLDDDTAKSTGLYRVLNWYCITKEERHNATPNCDGIQFRKHYLSVNRSAIDCSSTSYEENYDWSANALQVALNSWEDKKPKKLESAGSDKNCNIGQSSESHPCTMTEEWQTHYKETIEKLRELEEAYQRGKKAHDDMLGYANTAYAVNTKVEQEKPLSEV

SEQ ID NO: 9 - DNA, 1104 bp, synthetic construct
  source 1..1104: mol_type = other DNA
atgggcagcagccatcatcatcatcatcacagcagcggcctggtgccgcgcggcagccatatgctgctggtgattggcagcgaagataaccgcgtgccgggcgataaaaaactgaccaaagaaggcgcggcggcgctgtgcaaaatgaaacatctggcggataaagtggcgaaagaacgcagccaagaactgaaagatcgcacgcagaactttgcgggctatattgaatttgaactgtatcgcattgattattggctggaaaaactgaacggcccgaaaggccgcaaagatggctatgcgaaactgagcgatagcgatattaaaaaagtgaaagaaatttttgaaaaagcgaaagatggcattaccaaacagctgccggaagcgaaaaaagcggcggaagaagcggaaaaactgcatcaagaagtgaaagaagcggcggaaaaagcgcgcggccaagatctggatgatgataccgcgaaaagcaccggcctgtatcgcgtgctgaactggtattgcattaccaaagaagaacgccataacgcgaccccgaactgcgatggcattcagtttcgcaaacattatctgagcgtgaaccgcagcgcgattgattgcagcagcacgagctatgaagaaaactatgattggagcgcgaacgcgctgcaagtggcgctgaacagctgggaagataaaaaaccgaaaaaactggaaagcgcgggcagcgataaaaactgcaacattggtcagagcagcgaaagccatccgtgcaccatgaccgaagaatggcagacccattataaagaaaccattgaaaaactgcgcgaactggaagaagcgtatcagcgcggcaaaaaagcgcatgatgatatgctgggctatgcgaacaccgcgtatgcggtgaacaccaaagtggaacaagaaaaaccgctgagcgaagtgattgcggcggcgaaagaagcgggcaaaaaaggcgcgaaaattattattccggcggcggcgccggcgaccccgaccaacagcaccaaaaacgatgatagcgcgccgaccgaacatgtggatcgcggcattgcgaccaacgaaacccaagtggaagtgggcattgattaa

SEQ ID NO: 10 - protein, 367 aa, synthetic construct
MGSSHHHHHHSSGLVPRGSHMLLVIGSEDNRVPGDKKLTKEGAAALCKMKHLADKVAKERSQELKDRTQNFAGYIEFELYRIDYWLEKLNGPKGRKDGYAKLSDSDIKKVKEIFEKAKDGITKQLPEAKKAAEEAEKLHQEVKEAAEKARGQDLDDDTAKSTGLYRVLNWYCITKEERHNATPNCDGIQFRKHYLSVNRSAIDCSSTSYEENYDWSANALQVALNSWEDKKPKKLESAGSDKNCNIGQSSESHPCTMTEEWQTHYKETIEKLRELEEAYQRGKKAHDDMLGYANTAYAVNTKVEQEKPLSEVIAAAKEAGKKGAKIIIPAAAPATPTNSTKNDDSAPTEHVDRGIATNETQVEVGID

SEQ ID NO: 11 - protein, 21 aa, synthetic construct
MGSSHHHHHHSSGLVPRGSHM